European Patent Application EP 4 613 767 A1, published September 10, 2025. Title: 一种针对磷脂酰肌醇蛋白聚糖3的双特异性抗体及其应用. Applicant: 上海齐鲁制药研究中心有限公司. The sequence listing filed with the application follows.

SEQUENCE LISTING (18 sequences)

SEQ ID NO: 1 - protein, 125 aa, synthetic construct
EVKLVESGGGLVQPGGSLKLSCAASGFTFNTYAMNWVRQAPGKGLEWVARIRSKYNNYATYYADSVKDRFTISRDDAKNTLYLQMNNLRTEDTAVYYCVRHGNFGNSYVSWFAYWGQGTLVTVSS

SEQ ID NO: 2 - protein, 109 aa, synthetic construct
QAVVTQEPSLTVSPGGTVTLTCRSSTGAVTTSNYANWVQQKPGQAPRGLIGGTNKRAPGTPARFSGSLLGGKAALTLSGAQPEDEAEYYCALWYSNLWVFGGGTKLTVL

SEQ ID NO: 3 - protein, 250 aa, synthetic construct
EVKLVESGGGLVQPGGSLKLSCAASGFTFNTYAMNWVRQAPGKGLEWVARIRSKYNNYATYYADSVKDRFTISRDDAKNTLYLQMNNLRTEDTAVYYCVRHGNFGNSYVSWFAYWGQGTLVTVSSGGGGSGGGGSGGGGSAQAVVTQEPSLTVSPGGTVTLTCRSSTGAVTTSNYANWVQQKPGQAPRGLIGGTNKRAPGTPARFSGSLLGGKAALTLSGAQPEDEAEYYCALWYSNLWVFGGGTKLTVL

SEQ ID NO: 4 - protein, 5 aa, synthetic construct
TYAMN

SEQ ID NO: 5 - protein, 19 aa, synthetic construct
RIRSKYNNYATYYADSVKD

SEQ ID NO: 6 - protein, 14 aa, synthetic construct
HGNFGNSYVSWFAY

SEQ ID NO: 7 - protein, 14 aa, synthetic construct
RSSTGAVTTSNYAN

SEQ ID NO: 8 - protein, 7 aa, synthetic construct
GTNKRAP

SEQ ID NO: 9 - protein, 9 aa, synthetic construct
ALWYSNLWV

SEQ ID NO: 10 - protein, 121 aa, synthetic construct
QVQLVESGGGVVQPGGSLRLSCAASGRTLTNYVMGWFRQAPGKEREIVAGINWAGSRIGYGDFVKGRFTISRDNSKNTVYLQMNSLRPEDTAVYYCAAKLGKYNYPEYDYRGQGTLVTVSS

SEQ ID NO: 11 - protein, 5 aa, synthetic construct
NYVMG

SEQ ID NO: 12 - protein, 17 aa, synthetic construct
GINWAGSRIGYGDFVKG

SEQ ID NO: 13 - protein, 12 aa, synthetic construct
KLGKYNYPEYDY

SEQ ID NO: 14 - protein, 217 aa, synthetic construct
APEAAGGPSVFLFPPKPKDTLMISRTPEVTCVVVDVSHEDPEVKFNWYVDGVEVHNAKTKPREEQYNSTYRVVSVLTVLHQDWLNGKEYKCKVSNKALPAPIEKTISKAKGQPREPQVYTLPPCRDELTKNQVSLWCLVKGFYPSDIAVEWESNGQPENNYKTTPPVLDSDGSFFLYSKLTVDKSRWQQGNVFSCSVMHEALHNHYTQKSLSLSPGK

SEQ ID NO: 15 - protein, 217 aa, synthetic construct
APEAAGGPSVFLFPPKPKDTLMISRTPEVTCVVVDVSHEDPEVKFNWYVDGVEVHNAKTKPREEQYNSTYRVVSVLTVLHQDWLNGKEYKCKVSNKALPAPIEKTISKAKGQPREPQVCTLPPSRDELTKNQVSLSCAVKGFYPSDIAVEWESNGQPENNYKTTPPVLDSDGSFFLVSKLTVDKSRWQQGNVFSCSVMHEALHNRYTQKSLSLSPGK

SEQ ID NO: 16 - protein, 353 aa, synthetic construct
QVQLVESGGGVVQPGGSLRLSCAASGRTLTNYVMGWFRQAPGKEREIVAGINWAGSRIGYGDFVKGRFTISRDNSKNTVYLQMNSLRPEDTAVYYCAAKLGKYNYPEYDYRGQGTLVTVSSEPKSSDKTHTCPPCPAPEAAGGPSVFLFPPKPKDTLMISRTPEVTCVVVDVSHEDPEVKFNWYVDGVEVHNAKTKPREEQYNSTYRVVSVLTVLHQDWLNGKEYKCKVSNKALPAPIEKTISKAKGQPREPQVYTLPPCRDELTKNQVSLWCLVKGFYPSDIAVEWESNGQPENNYKTTPPVLDSDGSFFLYSKLTVDKSRWQQGNVFSCSVMHEALHNHYTQKSLSLSPGK

SEQ ID NO: 17 - protein, 482 aa, synthetic construct
EVKLVESGGGLVQPGGSLKLSCAASGFTFNTYAMNWVRQAPGKGLEWVARIRSKYNNYATYYADSVKDRFTISRDDAKNTLYLQMNNLRTEDTAVYYCVRHGNFGNSYVSWFAYWGQGTLVTVSSGGGGSGGGGSGGGGSAQAVVTQEPSLTVSPGGTVTLTCRSSTGAVTTSNYANWVQQKPGQAPRGLIGGTNKRAPGTPARFSGSLLGGKAALTLSGAQPEDEAEYYCALWYSNLWVFGGGTKLTVLEPKSSDKTHTCPPCPAPEAAGGPSVFLFPPKPKDTLMISRTPEVTCVVVDVSHEDPEVKFNWYVDGVEVHNAKTKPREEQYNSTYRVVSVLTVLHQDWLNGKEYKCKVSNKALPAPIEKTISKAKGQPREPQVCTLPPSRDELTKNQVSLSCAVKGFYPSDIAVEWESNGQPENNYKTTPPVLDSDGSFFLVSKLTVDKSRWQQGNVFSCSVMHEALHNRYTQKSLSLSPGK

SEQ ID NO: 18 - protein, 479 aa, synthetic construct
QVQLVESGGGVVQPGGSLRLSCAASGRTLTNYVMGWFRQAPGKEREIVAGINWAGSRIGYGDFVKGRFTISRDNSKNTVYLQMNSLRPEDTAVYYCAAKLGKYNYPEYDYRGQGTLVTVSSEPKSSDKTHTCPPCPAPEAAGGPSVFLFPPKPKDTLMISRTPEVTCVVVDVSHEDPEVKFNWYVDGVEVHNAKTKPREEQYNSTYRVVSVLTVLHQDWLNGKEYKCKVSNKALPAPIEKTISKAKGQPREPQVYTLPPCRDELTKNQVSLWCLVKGFYPSDIAVEWESNGQPENNYKTTPPVLDSDGSFFLYSKLTVDKSRWQQGNVFSCSVMHEALHNHYTQKSLSLSPGAGGGGSQVQLVESGGGVVQPGGSLRLSCAASGRTLTNYVMGWFRQAPGKEREIVAGINWAGSRIGYGDFVKGRFTISRDNSKNTVYLQMNSLRPEDTAVYYCAAKLGKYNYPEYDYRGQGTLVTVSS